European Patent Specification EP 3 950 942 B1, published April 29, 2026. Title: METHOD FOR PRODUCING KNOCK-IN CELL. Applicant: Osaka University. The sequence listing filed with the application follows.

SEQUENCE LISTING (24 sequences)

SEQ ID NO: 1 - DNA, 20 bp, Artificial Sequence
  primer sequence
actctgacagatgccaggac

SEQ ID NO: 2 - DNA, 20 bp, Artificial Sequence
  primer sequence
attctttctgacccggcaga

SEQ ID NO: 3 - DNA, 26 bp, Artificial Sequence
  primer sequence
gcgtgcacccgagtgtggtacttaag

SEQ ID NO: 4 - DNA, 24 bp, Artificial Sequence
  primer sequence
tccagggttctcctccacgtctcc

SEQ ID NO: 5 - DNA, 20 bp, Artificial Sequence
  primer sequence
ctgtccagcaccctgaagtc

SEQ ID NO: 6 - DNA, 20 bp, Artificial Sequence
  primer sequence
ggcacaacttctgttgaggc

SEQ ID NO: 7 - DNA, 20 bp, Artificial Sequence
  primer sequence
actctgacagatgccaggac

SEQ ID NO: 8 - DNA, 20 bp, Artificial Sequence
  primer sequence
attctttctgacccggcaga

SEQ ID NO: 9 - DNA, 20 bp, Artificial Sequence
  primer sequence
agctgtctggctagaatgag

SEQ ID NO: 10 - DNA, 24 bp, Artificial Sequence
  primer sequence
tccagggttctcctccacgtctcc

SEQ ID NO: 11 - DNA, 20 bp, Artificial Sequence
  primer sequence
ctgtccagcaccctgaagtc

SEQ ID NO: 12 - DNA, 23 bp, Artificial Sequence
  primer sequence
aggcttggctgttcattcttgta

SEQ ID NO: 13 - DNA, 20 bp, Artificial Sequence
  primer sequence
ggcaagctgaccctgaagtt

SEQ ID NO: 14 - DNA, 20 bp, Artificial Sequence
  primer sequence
tctcgttggggtctttgctc

SEQ ID NO: 15 - DNA, 20 bp, Artificial Sequence
  primer sequence
acctccacacttgtcttggc

SEQ ID NO: 16 - DNA, 20 bp, Artificial Sequence
  primer sequence
ccgcctcgccataaaaggaa

SEQ ID NO: 17 - DNA, 20 bp, Artificial Sequence
  primer sequence
ggcaagctgaccctgaagtt

SEQ ID NO: 18 - DNA, 20 bp, Artificial Sequence
  primer sequence
caccgtcaccatcagagcaa

SEQ ID NO: 19 - DNA, 23 bp, Artificial Sequence
  guide RNA sequence
gtataaatgactgcttaatgtgg

SEQ ID NO: 20 - DNA, 21 bp, Artificial Sequence
  guide RNA sequence
aaaggactatagatcataagg

SEQ ID NO: 21 - DNA, 23 bp, Artificial Sequence
  guide RNA sequence
gacatagggctagtctacaaagg

SEQ ID NO: 22 - DNA, 23 bp, Artificial Sequence
  guide RNA sequence
cggagacatggcgtaaagccagg

SEQ ID NO: 23 - DNA, 23 bp, Artificial Sequence
  guide RNA sequence
ccctgccagatagtccaccttct

SEQ ID NO: 24 - DNA, 23 bp, Artificial Sequence
  guide RNA sequence
ccacagcgacagggtcacctaat